European Patent Application EP 4 393 950 A1, published July 3, 2024. Title: FAP/CD40 BINDING MOLECULE AND MEDICINAL USE THEREOF. Applicant: JIANGSU HENGRUI PHARMACEUTICALS CO., LTD. Application CN PCT/CN2022/114522, filed August 24, 2022. The sequence listing filed with the application follows.

SEQUENCE LISTING (65 sequences)

SEQ ID NO: 1 - protein, 125 aa, Artificial sequence
QMQLVQSGAEVKKPGASVTVSCRASGYSFADHFIHWVRQAPGQGFQWMGWINPNRGVTHHAQDFQGRVAMTRDMSTDTVYMELTSLRSDDTAVYYCARDESLTARPYYFYGFDVWGQGTLVTVSS

SEQ ID NO: 2 - protein, 107 aa, Artificial sequence
DIQMTQSPSSVSASVGDRVTITCRASQGISSWLAWYQQKPGKAPKLLIYAASSLQSGVPSRFSGSGSGTDFTLTISSLQPEDFATYYCQQANSFPPAFGQGTKVEIK

SEQ ID NO: 3 - protein, 125 aa, Artificial sequence
QVQLQQSGVEVKKPGASVTVSCRASGYSFADHFIHWVRQAPGQGFQWMGWINPNRGVTHHAQDFQGRVAMTRDMSTDTVYMELTSLRSDDTAVYYCARDASLTARPYYFYGFDVWGQGTLVTVSS

SEQ ID NO: 4 - protein, 107 aa, Artificial sequence; identical to SEQ ID NO: 2

SEQ ID NO: 5 - protein, 125 aa, Artificial sequence; identical to SEQ ID NO: 3

SEQ ID NO: 6 - protein, 107 aa, Artificial sequence
EIVLTQSPSSVSASVGDRVTITCRASQGISSWLAWYQQKPGKAPKLLIYAASSLQSGVPSRFSGSGSGTDFTLTISSLQPEDFATYYCQQANSFPLTFGGGTKVEIK

SEQ ID NO: 7 - protein, 125 aa, Artificial sequence; identical to SEQ ID NO: 1

SEQ ID NO: 8 - protein, 107 aa, Artificial sequence
EIVLTQSPSSVSASVGDRVTITCRASQGISSWLAWYQQKPGKAPKSLIYAASSLQSGVPSRFSGSGSGTDFTLTISSLQPEDFATYYCQQANSFPPTFGGGTKVEIK

SEQ ID NO: 9 - protein, 5 aa, Artificial sequence
DHFIH

SEQ ID NO: 10 - protein, 17 aa, Artificial sequence
WINPNRGVTHHAQDFQG

SEQ ID NO: 11 - protein, 16 aa, Artificial sequence
DESLTARPYYFYGFDV

SEQ ID NO: 12 - protein, 11 aa, Artificial sequence
RASQGISSWLA

SEQ ID NO: 13 - protein, 6 aa, Artificial sequence
AASSLQ

SEQ ID NO: 14 - protein, 9 aa, Artificial sequence
QQANSFPPA

SEQ ID NO: 15 - protein, 16 aa, Artificial sequence
DASLTARPYYFYGFDV

SEQ ID NO: 16 - protein, 9 aa, Artificial sequence
QQANSFPLT

SEQ ID NO: 17 - protein, 9 aa, Artificial sequence
QQANSFPPT

SEQ ID NO: 18 - protein, 16 aa, Artificial sequence
  VARIANT 2: note = X can be E or A
DXSLTARPYYFYGFDV

SEQ ID NO: 19 - protein, 9 aa, Artificial sequence
  VARIANT 8: note = X can be P or L
  VARIANT 9: note = X can be A or T
QQANSFPXX

SEQ ID NO: 20 - protein, 116 aa, Artificial sequence
EVQLLESGGGLVQPGGSLRLSCAASGFTFSSHAMSWVRQAPGKGLEWVSAIWASGEQYYADSVKGRFTISRDNSKNTLYLQMNSLRAEDTAVYYCAKGWLGNFDYWGQGTLVTVSS

SEQ ID NO: 21 - protein, 108 aa, Artificial sequence
EIVLTQSPGTLSLSPGERATLSCRASQSVSRSYLAWYQQKPGQAPRLLIIGASTRATGIPDRFSGSGSGTDFTLTISRLEPEDFAVYYCQQGQVIPPTFGQGTKVEIK

SEQ ID NO: 22 - protein, 117 aa, Artificial sequence
EVQVVESGGGLAQPGGSLRLSCAASGFTFSNYGMKWVRQAPGKGPEWVSTILSQGGSTYYADSVKGRFTISRDNAKNTLYLQMNSLKPEDTALYYCLRVDWSDYSPRGQGTQVTVSA

SEQ ID NO: 23 - protein, 117 aa, Artificial sequence
QVQLVESGGGMVEPGGSLRLSCAASGFTFSRYGMKWVRQAPGKGPEWVSTINSHGDTTYYADSVKGRFTISRDNAQNTVYLQMNSLKPEDTALYYCLRIDYSDYSSRGQGTQVTVSS

SEQ ID NO: 24 - protein, 5 aa, Artificial sequence
NYGMK

SEQ ID NO: 25 - protein, 17 aa, Artificial sequence
TILSQGGSTYYADSVKG

SEQ ID NO: 26 - protein, 8 aa, Artificial sequence
VDWSDYSP

SEQ ID NO: 27 - protein, 5 aa, Artificial sequence
RYGMK

SEQ ID NO: 28 - protein, 17 aa, Artificial sequence
TINSHGDTTYYADSVKG

SEQ ID NO: 29 - protein, 8 aa, Artificial sequence
IDYSDYSS

SEQ ID NO: 30 - protein, 349 aa, Artificial sequence
EVQVVESGGGLAQPGGSLRLSCAASGFTFSNYGMKWVRQAPGKGPEWVSTILSQGGSTYYADSVKGRFTISRDNAKNTLYLQMNSLKPEDTALYYCLRVDWSDYSPRGQGTQVTVSAEPKSADKTHTCPPCPAPELLGGPSVFLFPPKPKDTLMISRTPEVTCVVVDVSHEDPEVKFNWYVDGVEVHNAKTKPREEQYASTYRVVSVLTVLHQDWLNGKEYKCKVSNKALPAPIEKTISKAKGQPREPQVYTLPPSREEMTKNQVSLTCLVKGFYPSDIAVEWESNGQPENNYKTTPPVLDSDGSFFLYSKLTVDKSRWQQGNVFSCSVMHEALHNHYTQKSLSLSPGK

SEQ ID NO: 31 - protein, 349 aa, Artificial sequence
QVQLVESGGGMVEPGGSLRLSCAASGFTFSRYGMKWVRQAPGKGPEWVSTINSHGDTTYYADSVKGRFTISRDNAQNTVYLQMNSLKPEDTALYYCLRIDYSDYSSRGQGTQVTVSSEPKSADKTHTCPPCPAPELLGGPSVFLFPPKPKDTLMISRTPEVTCVVVDVSHEDPEVKFNWYVDGVEVHNAKTKPREEQYASTYRVVSVLTVLHQDWLNGKEYKCKVSNKALPAPIEKTISKAKGQPREPQVYTLPPSREEMTKNQVSLTCLVKGFYPSDIAVEWESNGQPENNYKTTPPVLDSDGSFFLYSKLTVDKSRWQQGNVFSCSVMHEALHNHYTQKSLSLSPGK

SEQ ID NO: 32 - protein, 117 aa, Artificial sequence
EVQLVESGGGLVQPGGSLRLSCAASGFTFSNYGMKWVRQAPGKGLEWVSTILSQGGSTYYADSVKGRFTISRDNAKNSLYLQMNSLRAEDTALYYCARVDWSDYSPRGQGTMVTVSS

SEQ ID NO: 33 - protein, 117 aa, Artificial sequence
EVQLVESGGGLVQPGGSLRLSCAASGFTFSNYGMKWVRQAPGKGLEWVSTILSQGGSTYYADSVKGRFTISRDNAKNSLYLQMNSLRAEDTALYYCLRVDWSDYSPRGQGTQVTVSS

SEQ ID NO: 34 - protein, 117 aa, Artificial sequence
EVQVVESGGGLVQPGGSLRLSCAASGFTFSNYGMKWVRQAPGKGLEWVSTILSQGGSTYYADSVKGRFTISRDNSKNTLYLQMNSLRAEDTAVYYCLRVDWSDYSPRGQGTQVTVSS

SEQ ID NO: 35 - protein, 117 aa, Artificial sequence
QVQLVESGGGVVQPGGSLRLSCAASGFTFSRYGMKWVRQAPGKGLEWVSTINSHGDTTYYADSVKGRFTISRDNAKNSLYLQMNSLRAEDTALYYCARIDYSDYSSRGQGTMVTVSS

SEQ ID NO: 36 - protein, 117 aa, Artificial sequence
QVQLVESGGGVVQPGGSLRLSCAASGFTFSRYGMKWVRQAPGKGLEWVSTINSHGDTTYYADSVKGRFTISRDNAKNSLYLQMNSLRAEDTALYYCLRIDYSDYSSRGQGTMVTVSS

SEQ ID NO: 37 - protein, 117 aa, Artificial sequence
EVQLVESGGGLVQPGGSLRLSCAASGFTFSRYGMKWVRQAPGKGLEWVSTINSHGDTTYYADSVKGRFTISRDNAKNSLYLQMNSLRAEDTAVYYCLRIDYSDYSSRGQGTLVTVSS

SEQ ID NO: 38 - protein, 117 aa, Artificial sequence
EVQLVESGGGLVQPGGSLRLSCAASGFTFSRYGMKWVRQAPGKGLEWVSTINSHGDSTYYADSVKGRFTISRDNSKNTLYLQMNSLRAEDTAVYYCLKIDYSDYSSRGQGTLVTVSS

SEQ ID NO: 39 - protein, 5 aa, Artificial sequence
  VARIANT 1: note = X can be N or R
XYGMK

SEQ ID NO: 40 - protein, 17 aa, Artificial sequence
  VARIANT 3: note = X can be N or L
  VARIANT 5: note = X can be Q or H
  VARIANT 7: note = X can be G or D
  VARIANT 8: note = X can be S or T
TIXSXGXXTYYADSVKG

SEQ ID NO: 41 - protein, 8 aa, Artificial sequence
  VARIANT 1: note = X can be V or I
  VARIANT 3: note = X can be W or Y
  VARIANT 8: note = X can be P or S
XDXSDYSX

SEQ ID NO: 42 - protein, 582 aa, Artificial sequence
QVQLQQSGVEVKKPGASVTVSCRASGYSFADHFIHWVRQAPGQGFQWMGWINPNRGVTHHAQDFQGRVAMTRDMSTDTVYMELTSLRSDDTAVYYCARDASLTARPYYFYGFDVWGQGTLVTVSSASTKGPSVFPLAPSSKSTSGGTAALGCLVKDYFPEPVTVSWNSGALTSGVHTFPAVLQSSGLYSLSSVVTVPSSSLGTQTYICNVNHKPSNTKVDKKVEPKSCDKTHTCPPCPAPEAAGGPSVFLFPPKPKDTLMISRTPEVTCVVVDVSHEDPEVKFNWYVDGVEVHNAKTKPREEQYNSTYRVVSVLTVLHQDWLNGKEYKCKVSNKALPAPIEKTISKAKGQPREPQVYTLPPSRDELTKNQVSLTCLVKGFYPSDIAVEWESNGQPENNYKTTPPVLDSDGSFFLYSKLTVDKSRWQQGNVFSCSVMHEALHNHYTQKSLSLSPGKGGGGSGGGGSEVQLVESGGGLVQPGGSLRLSCAASGFTFSNYGMKWVRQAPGKGLEWVSTILSQGGSTYYADSVKGRFTISRDNAKNSLYLQMNSLRAEDTALYYCLRVDWSDYSPRGQGTQVTVSS

SEQ ID NO: 43 - protein, 214 aa, Artificial sequence
DIQMTQSPSSVSASVGDRVTITCRASQGISSWLAWYQQKPGKAPKLLIYAASSLQSGVPSRFSGSGSGTDFTLTISSLQPEDFATYYCQQANSFPPAFGQGTKVEIKRTVAAPSVFIFPPSDEQLKSGTASVVCLLNNFYPREAKVQWKVDNALQSGNSQESVTEQDSKDSTYSLSSTLTLSKADYEKHKVYACEVTHQGLSSPVTKSFNRGEC

SEQ ID NO: 44 - protein, 709 aa, Artificial sequence
QVQLQQSGVEVKKPGASVTVSCRASGYSFADHFIHWVRQAPGQGFQWMGWINPNRGVTHHAQDFQGRVAMTRDMSTDTVYMELTSLRSDDTAVYYCARDASLTARPYYFYGFDVWGQGTLVTVSSASTKGPSVFPLAPSSKSTSGGTAALGCLVKDYFPEPVTVSWNSGALTSGVHTFPAVLQSSGLYSLSSVVTVPSSSLGTQTYICNVNHKPSNTKVDKKVEPKSCDKTHTCPPCPAPEAAGGPSVFLFPPKPKDTLMISRTPEVTCVVVDVSHEDPEVKFNWYVDGVEVHNAKTKPREEQYNSTYRVVSVLTVLHQDWLNGKEYKCKVSNKALPAPIEKTISKAKGQPREPQVYTLPPSRDELTKNQVSLTCLVKGFYPSDIAVEWESNGQPENNYKTTPPVLDSDGSFFLYSKLTVDKSRWQQGNVFSCSVMHEALHNHYTQKSLSLSPGKGGGGSGGGGSEVQLVESGGGLVQPGGSLRLSCAASGFTFSNYGMKWVRQAPGKGLEWVSTILSQGGSTYYADSVKGRFTISRDNAKNSLYLQMNSLRAEDTALYYCLRVDWSDYSPRGQGTQVTVSSGGGGSGGGGSEVQLVESGGGLVQPGGSLRLSCAASGFTFSNYGMKWVRQAPGKGLEWVSTILSQGGSTYYADSVKGRFTISRDNAKNSLYLQMNSLRAEDTALYYCLRVDWSDYSPRGQGTQVTVSS

SEQ ID NO: 45 - protein, 836 aa, Artificial sequence
QVQLQQSGVEVKKPGASVTVSCRASGYSFADHFIHWVRQAPGQGFQWMGWINPNRGVTHHAQDFQGRVAMTRDMSTDTVYMELTSLRSDDTAVYYCARDASLTARPYYFYGFDVWGQGTLVTVSSASTKGPSVFPLAPSSKSTSGGTAALGCLVKDYFPEPVTVSWNSGALTSGVHTFPAVLQSSGLYSLSSVVTVPSSSLGTQTYICNVNHKPSNTKVDKKVEPKSCDKTHTCPPCPAPEAAGGPSVFLFPPKPKDTLMISRTPEVTCVVVDVSHEDPEVKFNWYVDGVEVHNAKTKPREEQYNSTYRVVSVLTVLHQDWLNGKEYKCKVSNKALPAPIEKTISKAKGQPREPQVYTLPPSRDELTKNQVSLTCLVKGFYPSDIAVEWESNGQPENNYKTTPPVLDSDGSFFLYSKLTVDKSRWQQGNVFSCSVMHEALHNHYTQKSLSLSPGKGGGGSGGGGSEVQLVESGGGLVQPGGSLRLSCAASGFTFSNYGMKWVRQAPGKGLEWVSTILSQGGSTYYADSVKGRFTISRDNAKNSLYLQMNSLRAEDTALYYCLRVDWSDYSPRGQGTQVTVSSGGGGSGGGGSEVQLVESGGGLVQPGGSLRLSCAASGFTFSNYGMKWVRQAPGKGLEWVSTILSQGGSTYYADSVKGRFTISRDNAKNSLYLQMNSLRAEDTALYYCLRVDWSDYSPRGQGTQVTVSSGGGGSGGGGSEVQLVESGGGLVQPGGSLRLSCAASGFTFSNYGMKWVRQAPGKGLEWVSTILSQGGSTYYADSVKGRFTISRDNAKNSLYLQMNSLRAEDTALYYCLRVDWSDYSPRGQGTQVTVSS

SEQ ID NO: 46 - protein, 582 aa, Artificial sequence
QVQLQQSGVEVKKPGASVTVSCRASGYSFADHFIHWVRQAPGQGFQWMGWINPNRGVTHHAQDFQGRVAMTRDMSTDTVYMELTSLRSDDTAVYYCARDASLTARPYYFYGFDVWGQGTLVTVSSASTKGPSVFPLAPSSKSTSGGTAALGCLVKDYFPEPVTVSWNSGALTSGVHTFPAVLQSSGLYSLSSVVTVPSSSLGTQTYICNVNHKPSNTKVDKKVEPKSCDKTHTCPPCPAPEAAGGPSVFLFPPKPKDTLMISRTPEVTCVVVDVSHEDPEVKFNWYVDGVEVHNAKTKPREEQYNSTYRVVSVLTVLHQDWLNGKEYKCKVSNKALPAPIEKTISKAKGQPREPQVYTLPPSRDELTKNQVSLTCLVKGFYPSDIAVEWESNGQPENNYKTTPPVLDSDGSFFLYSKLTVDKSRWQQGNVFSCSVMHEALHNHYTQKSLSLSPGKGGGGSGGGGSEVQLVESGGGLVQPGGSLRLSCAASGFTFSRYGMKWVRQAPGKGLEWVSTINSHGDTTYYADSVKGRFTISRDNAKNSLYLQMNSLRAEDTAVYYCLRIDYSDYSSRGQGTLVTVSS

SEQ ID NO: 47 - protein, 709 aa, Artificial sequence
QVQLQQSGVEVKKPGASVTVSCRASGYSFADHFIHWVRQAPGQGFQWMGWINPNRGVTHHAQDFQGRVAMTRDMSTDTVYMELTSLRSDDTAVYYCARDASLTARPYYFYGFDVWGQGTLVTVSSASTKGPSVFPLAPSSKSTSGGTAALGCLVKDYFPEPVTVSWNSGALTSGVHTFPAVLQSSGLYSLSSVVTVPSSSLGTQTYICNVNHKPSNTKVDKKVEPKSCDKTHTCPPCPAPEAAGGPSVFLFPPKPKDTLMISRTPEVTCVVVDVSHEDPEVKFNWYVDGVEVHNAKTKPREEQYNSTYRVVSVLTVLHQDWLNGKEYKCKVSNKALPAPIEKTISKAKGQPREPQVYTLPPSRDELTKNQVSLTCLVKGFYPSDIAVEWESNGQPENNYKTTPPVLDSDGSFFLYSKLTVDKSRWQQGNVFSCSVMHEALHNHYTQKSLSLSPGKGGGGSGGGGSEVQLVESGGGLVQPGGSLRLSCAASGFTFSRYGMKWVRQAPGKGLEWVSTINSHGDTTYYADSVKGRFTISRDNAKNSLYLQMNSLRAEDTAVYYCLRIDYSDYSSRGQGTLVTVSSGGGGSGGGGSEVQLVESGGGLVQPGGSLRLSCAASGFTFSRYGMKWVRQAPGKGLEWVSTINSHGDTTYYADSVKGRFTISRDNAKNSLYLQMNSLRAEDTAVYYCLRIDYSDYSSRGQGTLVTVSS

SEQ ID NO: 48 - protein, 836 aa, Artificial sequence
QVQLQQSGVEVKKPGASVTVSCRASGYSFADHFIHWVRQAPGQGFQWMGWINPNRGVTHHAQDFQGRVAMTRDMSTDTVYMELTSLRSDDTAVYYCARDASLTARPYYFYGFDVWGQGTLVTVSSASTKGPSVFPLAPSSKSTSGGTAALGCLVKDYFPEPVTVSWNSGALTSGVHTFPAVLQSSGLYSLSSVVTVPSSSLGTQTYICNVNHKPSNTKVDKKVEPKSCDKTHTCPPCPAPEAAGGPSVFLFPPKPKDTLMISRTPEVTCVVVDVSHEDPEVKFNWYVDGVEVHNAKTKPREEQYNSTYRVVSVLTVLHQDWLNGKEYKCKVSNKALPAPIEKTISKAKGQPREPQVYTLPPSRDELTKNQVSLTCLVKGFYPSDIAVEWESNGQPENNYKTTPPVLDSDGSFFLYSKLTVDKSRWQQGNVFSCSVMHEALHNHYTQKSLSLSPGKGGGGSGGGGSEVQLVESGGGLVQPGGSLRLSCAASGFTFSRYGMKWVRQAPGKGLEWVSTINSHGDTTYYADSVKGRFTISRDNAKNSLYLQMNSLRAEDTAVYYCLRIDYSDYSSRGQGTLVTVSSGGGGSGGGGSEVQLVESGGGLVQPGGSLRLSCAASGFTFSRYGMKWVRQAPGKGLEWVSTINSHGDTTYYADSVKGRFTISRDNAKNSLYLQMNSLRAEDTAVYYCLRIDYSDYSSRGQGTLVTVSSGGGGSGGGGSEVQLVESGGGLVQPGGSLRLSCAASGFTFSRYGMKWVRQAPGKGLEWVSTINSHGDTTYYADSVKGRFTISRDNAKNSLYLQMNSLRAEDTAVYYCLRIDYSDYSSRGQGTLVTVSS

SEQ ID NO: 49 - protein, 455 aa, Artificial sequence
QMQLVQSGAEVKKPGASVTVSCRASGYSFADHFIHWVRQAPGQGFQWMGWINPNRGVTHHAQDFQGRVAMTRDMSTDTVYMELTSLRSDDTAVYYCARDESLTARPYYFYGFDVWGQGTLVTVSSASTKGPSVFPLAPSSKSTSGGTAALGCLVKDYFPEPVTVSWNSGALTSGVHTFPAVLQSSGLYSLSSVVTVPSSSLGTQTYICNVNHKPSNTKVDKKVEPKSCDKTHTCPPCPAPEAAGGPSVFLFPPKPKDTLMISRTPEVTCVVVDVSHEDPEVKFNWYVDGVEVHNAKTKPREEQYNSTYRVVSVLTVLHQDWLNGKEYKCKVSNKALPAPIEKTISKAKGQPREPQVYTLPPSRDELTKNQVSLTCLVKGFYPSDIAVEWESNGQPENNYKTTPPVLDSDGSFFLYSKLTVDKSRWQQGNVFSCSVMHEALHNHYTQKSLSLSPGK

SEQ ID NO: 50 - protein, 214 aa, Artificial sequence; identical to SEQ ID NO: 43

SEQ ID NO: 51 - protein, 455 aa, Artificial sequence
QVQLQQSGVEVKKPGASVTVSCRASGYSFADHFIHWVRQAPGQGFQWMGWINPNRGVTHHAQDFQGRVAMTRDMSTDTVYMELTSLRSDDTAVYYCARDASLTARPYYFYGFDVWGQGTLVTVSSASTKGPSVFPLAPSSKSTSGGTAALGCLVKDYFPEPVTVSWNSGALTSGVHTFPAVLQSSGLYSLSSVVTVPSSSLGTQTYICNVNHKPSNTKVDKKVEPKSCDKTHTCPPCPAPEAAGGPSVFLFPPKPKDTLMISRTPEVTCVVVDVSHEDPEVKFNWYVDGVEVHNAKTKPREEQYNSTYRVVSVLTVLHQDWLNGKEYKCKVSNKALPAPIEKTISKAKGQPREPQVYTLPPSRDELTKNQVSLTCLVKGFYPSDIAVEWESNGQPENNYKTTPPVLDSDGSFFLYSKLTVDKSRWQQGNVFSCSVMHEALHNHYTQKSLSLSPGK

SEQ ID NO: 52 - protein, 214 aa, Artificial sequence; identical to SEQ ID NO: 43

SEQ ID NO: 53 - protein, 455 aa, Artificial sequence; identical to SEQ ID NO: 51

SEQ ID NO: 54 - protein, 214 aa, Artificial sequence
EIVLTQSPSSVSASVGDRVTITCRASQGISSWLAWYQQKPGKAPKLLIYAASSLQSGVPSRFSGSGSGTDFTLTISSLQPEDFATYYCQQANSFPLTFGGGTKVEIKRTVAAPSVFIFPPSDEQLKSGTASVVCLLNNFYPREAKVQWKVDNALQSGNSQESVTEQDSKDSTYSLSSTLTLSKADYEKHKVYACEVTHQGLSSPVTKSFNRGEC

SEQ ID NO: 55 - protein, 455 aa, Artificial sequence; identical to SEQ ID NO: 49

SEQ ID NO: 56 - protein, 214 aa, Artificial sequence
EIVLTQSPSSVSASVGDRVTITCRASQGISSWLAWYQQKPGKAPKSLIYAASSLQSGVPSRFSGSGSGTDFTLTISSLQPEDFATYYCQQANSFPPTFGGGTKVEIKRTVAAPSVFIFPPSDEQLKSGTASVVCLLNNFYPREAKVQWKVDNALQSGNSQESVTEQDSKDSTYSLSSTLTLSKADYEKHKVYACEVTHQGLSSPVTKSFNRGEC

SEQ ID NO: 57 - protein, 349 aa, Artificial sequence
EVQLVESGGGLVQPGGSLRLSCAASGFTFSNYGMKWVRQAPGKGLEWVSTILSQGGSTYYADSVKGRFTISRDNAKNSLYLQMNSLRAEDTALYYCARVDWSDYSPRGQGTMVTVSSEPKSADKTHTCPPCPAPELLGGPSVFLFPPKPKDTLMISRTPEVTCVVVDVEHEDPEVKFNWYVDGVEVHNAKTKPREEQYNSTYRVVSVLTVLHQDWLNGKEYKCKVSSKAFPAPIEKTISKAKGQPREPQVYTLPPSRDELTKNQVSLTCLVKGFYPSDIAVEWESNGQPENNYKTTPPVLDSDGSFFLYSKLTVDKSRWQQGNVFSCSVMHEALHNHYTQKSLSLSPGK

SEQ ID NO: 58 - protein, 349 aa, Artificial sequence
EVQLVESGGGLVQPGGSLRLSCAASGFTFSNYGMKWVRQAPGKGLEWVSTILSQGGSTYYADSVKGRFTISRDNAKNSLYLQMNSLRAEDTALYYCLRVDWSDYSPRGQGTQVTVSSEPKSADKTHTCPPCPAPELLGGPSVFLFPPKPKDTLMISRTPEVTCVVVDVEHEDPEVKFNWYVDGVEVHNAKTKPREEQYNSTYRVVSVLTVLHQDWLNGKEYKCKVSSKAFPAPIEKTISKAKGQPREPQVYTLPPSRDELTKNQVSLTCLVKGFYPSDIAVEWESNGQPENNYKTTPPVLDSDGSFFLYSKLTVDKSRWQQGNVFSCSVMHEALHNHYTQKSLSLSPGK

SEQ ID NO: 59 - protein, 349 aa, Artificial sequence
EVQVVESGGGLVQPGGSLRLSCAASGFTFSNYGMKWVRQAPGKGLEWVSTILSQGGSTYYADSVKGRFTISRDNSKNTLYLQMNSLRAEDTAVYYCLRVDWSDYSPRGQGTQVTVSSEPKSADKTHTCPPCPAPELLGGPSVFLFPPKPKDTLMISRTPEVTCVVVDVEHEDPEVKFNWYVDGVEVHNAKTKPREEQYNSTYRVVSVLTVLHQDWLNGKEYKCKVSSKAFPAPIEKTISKAKGQPREPQVYTLPPSRDELTKNQVSLTCLVKGFYPSDIAVEWESNGQPENNYKTTPPVLDSDGSFFLYSKLTVDKSRWQQGNVFSCSVMHEALHNHYTQKSLSLSPGK

SEQ ID NO: 60 - protein, 349 aa, Artificial sequence
QVQLVESGGGVVQPGGSLRLSCAASGFTFSRYGMKWVRQAPGKGLEWVSTINSHGDTTYYADSVKGRFTISRDNAKNSLYLQMNSLRAEDTALYYCARIDYSDYSSRGQGTMVTVSSEPKSADKTHTCPPCPAPELLGGPSVFLFPPKPKDTLMISRTPEVTCVVVDVEHEDPEVKFNWYVDGVEVHNAKTKPREEQYNSTYRVVSVLTVLHQDWLNGKEYKCKVSSKAFPAPIEKTISKAKGQPREPQVYTLPPSRDELTKNQVSLTCLVKGFYPSDIAVEWESNGQPENNYKTTPPVLDSDGSFFLYSKLTVDKSRWQQGNVFSCSVMHEALHNHYTQKSLSLSPGK

SEQ ID NO: 61 - protein, 349 aa, Artificial sequence
QVQLVESGGGVVQPGGSLRLSCAASGFTFSRYGMKWVRQAPGKGLEWVSTINSHGDTTYYADSVKGRFTISRDNAKNSLYLQMNSLRAEDTALYYCLRIDYSDYSSRGQGTMVTVSSEPKSADKTHTCPPCPAPELLGGPSVFLFPPKPKDTLMISRTPEVTCVVVDVEHEDPEVKFNWYVDGVEVHNAKTKPREEQYNSTYRVVSVLTVLHQDWLNGKEYKCKVSSKAFPAPIEKTISKAKGQPREPQVYTLPPSRDELTKNQVSLTCLVKGFYPSDIAVEWESNGQPENNYKTTPPVLDSDGSFFLYSKLTVDKSRWQQGNVFSCSVMHEALHNHYTQKSLSLSPGK

SEQ ID NO: 62 - protein, 349 aa, Artificial sequence
EVQLVESGGGLVQPGGSLRLSCAASGFTFSRYGMKWVRQAPGKGLEWVSTINSHGDTTYYADSVKGRFTISRDNAKNSLYLQMNSLRAEDTAVYYCLRIDYSDYSSRGQGTLVTVSSEPKSADKTHTCPPCPAPELLGGPSVFLFPPKPKDTLMISRTPEVTCVVVDVEHEDPEVKFNWYVDGVEVHNAKTKPREEQYNSTYRVVSVLTVLHQDWLNGKEYKCKVSSKAFPAPIEKTISKAKGQPREPQVYTLPPSRDELTKNQVSLTCLVKGFYPSDIAVEWESNGQPENNYKTTPPVLDSDGSFFLYSKLTVDKSRWQQGNVFSCSVMHEALHNHYTQKSLSLSPGK

SEQ ID NO: 63 - protein, 349 aa, Artificial sequence
EVQLVESGGGLVQPGGSLRLSCAASGFTFSRYGMKWVRQAPGKGLEWVSTINSHGDSTYYADSVKGRFTISRDNSKNTLYLQMNSLRAEDTAVYYCLKIDYSDYSSRGQGTLVTVSSEPKSADKTHTCPPCPAPELLGGPSVFLFPPKPKDTLMISRTPEVTCVVVDVEHEDPEVKFNWYVDGVEVHNAKTKPREEQYNSTYRVVSVLTVLHQDWLNGKEYKCKVSSKAFPAPIEKTISKAKGQPREPQVYTLPPSRDELTKNQVSLTCLVKGFYPSDIAVEWESNGQPENNYKTTPPVLDSDGSFFLYSKLTVDKSRWQQGNVFSCSVMHEALHNHYTQKSLSLSPGK

SEQ ID NO: 64 - protein, 436 aa, Artificial sequence
QVQLVQSGAEVKKPGASVKVSCKASGYILTTYWITWVRQAPGQGLEWMGDIHPGSGSTKYNEKFKSRVTLTVDTSISTAYMELSRLRSEDTAVYYCARRDYWGQGTTVTVSSAKTTPPSVYPLAPGSAAQTNSMVTLGCLVKGYFPEPVTVTWNSGSLSSGVHTFPAVLQSDLYTLSSSVTVPSSTWPSETVTCNVAHPASSTKVDKKIVPRDCGCKPCICTVPEVSSVFIFPPKPKDVLTITLTPKVTCVVVDISKDDPEVQFSWFVDDVEVHTAQTQPREEQFNSTFRSVSELPIMHQDWLNGKEFKCRVNSAAFPAPIEKTISKTKGRPKAPQVYTIPPPKEQMAKDKVSLTCMITDFFPEDITVEWQWNGQPAENYKNTQPIMDTDGSYFVYSKLNVQKSNWEAGNTFTCSVLHEGLHNHHTEKSLSHSPGK

SEQ ID NO: 65 - protein, 219 aa, Artificial sequence
DIVMTQSPLSLPVTPGEPASISCRSSQNIVNSQGNTYLEWYLQKPGQSPQLLIYKVTNRFSGVPDRFSGSGSGTDFTLKISRVEAEDVGVYYCFQASLVPWTFGGGTKVEIKRADAAPTVSIFPPSSEQLTSGGASVVCFLNNFYPKDINVKWKIDGSERQNGVLNSWTDQDSKDSTYSMSSTLTLTKDEYERHNSYTCEATHKTSTSPIVKSFNRNEC